European Patent Specification EP 3 702 461 B1, published September 9, 2026. Title: METHODS FOR PERFORMING ANTISENSE OLIGONUCLEOTIDE-MEDIATED EXON SKIPPING IN THE RETINA OF A SUBJECT IN NEED THEREOF. Applicant: Institut National de la Santé et de la Recherche Médicale (INSERM) UNIVERSITE DE PARIS FONDATION IMAGINE Assistance Publique-Hôpitaux de Paris. The sequence listing filed with the application follows.

SEQUENCE LISTING (32 sequences)

SEQ ID NO: 1 - DNA, 20 bp, Artificial
  primer
gaccaccttgagaaggaaac

SEQ ID NO: 2 - DNA, 19 bp, Artificial
  primer
catcctgctcagcttgatc

SEQ ID NO: 3 - DNA, 20 bp, Artificial
  primer
cccaccaaactattgccaac

SEQ ID NO: 4 - DNA, 22 bp, Artificial
  primer
gagagtcatcttgttctgctac

SEQ ID NO: 5 - DNA, 26 bp, Artificial
  primer
tgactgctaagtacagggacatcttg

SEQ ID NO: 6 - DNA, 24 bp, Artificial
  primer
aggagatgttttcacactccaggt

SEQ ID NO: 7 - DNA, 23 bp, Artificial
  primer
ctggccccagttgtaatttgtga

SEQ ID NO: 8 - DNA, 24 bp, Artificial
  primer
ctgttcccaggcttgttcaatagt

SEQ ID NO: 9 - DNA, 24 bp, Artificial
  primer
tgactgctaagtacagggacatct

SEQ ID NO: 10 - DNA, 24 bp, Artificial
  primer
aggagatgttttcacactccaggt

SEQ ID NO: 11 - DNA, 23 bp, Artificial
  primer
ctggccccagttgtaatttgtga

SEQ ID NO: 12 - DNA, 24 bp, Artificial
  primer
ctgttcccaggcttgttcaatagt

SEQ ID NO: 13 - DNA, 25 bp, Artificial
  primer
tgacctaaagaccattgcacttcgt

SEQ ID NO: 14 - DNA, 20 bp, Artificial
  primer
ctgcagcaaatcgcttggga

SEQ ID NO: 15 - DNA, 25 bp, Artificial
  primer
cctgtatgctatccagaaaacccct

SEQ ID NO: 16 - DNA, 25 bp, Artificial
  primer
cgtagcagttcagtatgttcggctt

SEQ ID NO: 17 - DNA, 22 bp, Artificial
  primer
ctgcggttgtgatgtggtctgt

SEQ ID NO: 18 - DNA, 24 bp, Artificial
  primer
tgtgggtgatcagcgtcttaaagt

SEQ ID NO: 19 - DNA, 24 bp, Artificial
  primer
gttggatacaggccagactttgtt

SEQ ID NO: 20 - DNA, 25 bp, Artificial
  primer
aaacgtgattcaaatccctgaagta

SEQ ID NO: 21 - DNA, 22 bp, Artificial
  primer
ccaaacacaaacggttcccagt

SEQ ID NO: 22 - DNA, 20 bp, Artificial
  primer
gcttgccatccagccattca

SEQ ID NO: 23 - DNA, 25 bp, Artificial
  primer
gggacagtgagtacccagacatcta

SEQ ID NO: 24 - DNA, 22 bp, Artificial
  primer
ccagacttggtgttggatgctt

SEQ ID NO: 25 - DNA, 28 bp, Artificial
  Antisense
caaagaagtaccagatctggggccctac

SEQ ID NO: 26 - DNA, 21 bp, Artificial
  primer
tgatccagagcctggagtcaa

SEQ ID NO: 27 - DNA, 21 bp, Artificial
  primer
ttcttctccgagctgcctatt

SEQ ID NO: 28 - RNA, 30 nt, Artificial Sequence
  m23D(+11-18)
guuuucaaaauauaaauaccuuagguauuc

SEQ ID NO: 29 - RNA, 20 nt, Artificial Sequence
  m23ESE(+50+70)
gaugacgaaucacugcaaac

SEQ ID NO: 30 - RNA, 24 nt, Artificial Sequence
  m36D(+8-16)
guucucagaaucuuaccugagcug

SEQ ID NO: 31 - RNA, 20 nt, Artificial Sequence
  m36ESE(+23+44)
caugaaggucuuccucaugc

SEQ ID NO: 32 - RNA, 20 nt, Artificial Sequence
  m23ESEsense
guuugcagugauucgucauc